European Patent Specification EP 3 202 418 B1, published August 23, 2023. Title: CYTOTOXIC ANTI-LAG-3 MONOCLONAL ANTIBODY AND ITS USE IN THE TREATMENT OR PREVENTION OF ORGAN TRANSPLANT REJECTION AND AUTOIMMUNE DISEASE. Applicant: HAUDEBOURG, Thomas TRIEBEL, Frederic VANHOVE, Bernard. Application 12/598,128. The sequence listing filed with the application follows.

SEQUENCE LISTING (7 sequences)

SEQ ID NO: 1 - protein, 25 aa, Rattus norvegicus
DQPASIPALDLLQGMPSTRRHPPHR

SEQ ID NO: 2 - DNA, 28 bp, Artificial Sequence
  Primer
atatgaattcacagaggagatgaggcag

SEQ ID NO: 3 - DNA, 28 bp, Artificial Sequence
  Primer
atatgaattctcctggtcagagctgcct

SEQ ID NO: 4 - DNA, 21 bp, Artificial Sequence
  Primer
tggatgctatggaaggaaaga

SEQ ID NO: 5 - DNA, 20 bp, Artificial Sequence
  Primer
gattctggtgacagctggtg

SEQ ID NO: 6 - DNA, 21 bp, Artificial Sequence
  Primer
ccttggtcaagcagtacagcc

SEQ ID NO: 7 - DNA, 22 bp, Artificial Sequence
  Primer
ttcgctgatgacacaaacatga